European Patent Application EP 4 431 526 A1, published September 18, 2024. Title: Anti-GPVI antibodies and functional fragments thereof. Applicant: Emfret Analytics GmbH & CoKG (Eibelstadt). The sequence listing filed with the application follows.

SEQUENCE LISTING (63 sequences)

SEQ ID NO: 1 - protein, 11 aa, synthetic construct
KASQNVGTYVA

SEQ ID NO: 2 - protein, 7 aa, synthetic construct
SASYRCS

SEQ ID NO: 3 - protein, 9 aa, synthetic construct
HQYNNYPLT

SEQ ID NO: 4 - protein, 10 aa, synthetic construct
GFSLTSYGVT

SEQ ID NO: 5 - protein, 16 aa, synthetic construct
VIWGDGSTNYHSGLRS

SEQ ID NO: 6 - protein, 15 aa, synthetic construct
AKPIYYDFDDDAMDY

SEQ ID NO: 7 - protein, 6 aa, synthetic construct
QNVGTY

SEQ ID NO: 8 - protein, 5 aa, synthetic construct
SASYR

SEQ ID NO: 9 - protein, 7 aa, synthetic construct
  VARIANT 6: note = X is A, R, N, D, Q, E, G, H, I, L, K, M, F, S, T, W, Y, or V
SASYRXS

SEQ ID NO: 10 - protein, 5 aa, synthetic construct
SYGVT

SEQ ID NO: 11 - protein, 8 aa, synthetic construct
GFSLTSYG

SEQ ID NO: 12 - protein, 7 aa, synthetic construct
IWGDGST

SEQ ID NO: 13 - protein, 16 aa, synthetic construct
  VARIANT 5: note = X is A, R, N, D, Q, E, G, H, I, L, K, M, F, S, T, W, Y, or V
  VARIANT 6: note = X is A, R, N, D, Q, E, G, H, I, L, K, M, F, S, T, W, Y, or V
VIWGXXSTNYHSGLRS

SEQ ID NO: 14 - protein, 13 aa, synthetic construct
PIYYDFDDDAMDY

SEQ ID NO: 15 - protein, 107 aa, synthetic construct
DIVMTQSQKFMSTSVGDRVSVTCKASQNVGTYVAWFQQKPGQSPKTLIYSASYRCSGVPDRFTGSGSGTDFTLTISNVQSDDLAEYFCHQYNNYPLTFGAGTKLELR

SEQ ID NO: 16 - protein, 107 aa, synthetic construct
EIVLTQSPSSLSASVGDRVTITCKASQNVGTYVAWFQQKPGKAPKSLIYSASYRCSGVPSKFSGSGSGTDFTLTISSLQPEDFATYYCHQYNNYPLTFGQGTKLEIK

SEQ ID NO: 17 - protein, 107 aa, synthetic construct
DIQMTQSPSSLSASVGDRVTITCKASQNVGTYVAWFQQRPGKAPKSLIYSASYRCSGVPSKFSGSGSGTDFTLTINSLQPEDFATYYCHQYNNYPLTFGQGTKVEIK

SEQ ID NO: 18 - protein, 107 aa, synthetic construct
DIQLTQSPSTLSASVGDRVTITCKASQNVGTYVAWYQQKPGKAPKLLIYSASYRCSGVPSRFSGSGSGTEFTLTISSLQPDDFTTYYCHQYNNYPLTFGQGTKVEIK

SEQ ID NO: 19 - protein, 107 aa, synthetic construct
DIVMTQSPATLSLSPGDRATLSCKASQNVGTYVAWYQQKPGQAPRLLIYSASYRCSGIPARFSGSGSGTDFTLTISSLQSEDFAVYYCHQYNNYPLTFGGGTKVEIK

SEQ ID NO: 20 - protein, 121 aa, synthetic construct
QVQLKESGPGLVQPSQSLSITCTVSGFSLTSYGVTWVRQPPGKGLEWLGVIWGDGSTNYHSGLRSRLSISRDDSKSQVFLKLNSLQTDDTATYYCAKPIYYDFDDDAMDYWGQGTSVTVSS

SEQ ID NO: 21 - protein, 121 aa, synthetic construct
QVQLQESGPGLVKPSETLSLTCTASGFSLTSYGVTWIRQPPGKGLEWIGVIWGDGSTNYHSGLRSRVTISVDTSKSQFSLKLSSVTAADTAVYYCAKPIYYDFDDDAMDYWGQGTLVTVSS

SEQ ID NO: 22 - protein, 121 aa, synthetic construct
EVQLVESGPGLVKPSETLSLTCTVSGFSLTSYGVTWIRQPPGKGLEWIGVIWGDGSTNYHSGLRSRVTISVDTSKNQFSLKLSSVTAADTAVYYCAKPIYYDFDDDAMDYWGQGTLVTVSS

SEQ ID NO: 23 - protein, 121 aa, synthetic construct
QVQLVESGGGVVQPGRSLRLSCVASGFSLTSYGVTWVRQAPGKGLEWVAVIWGDGSTNYHSGLRSRFTISRDNSKNTMFLQMNSLRADDTAVYYCAKPIYYDFDDDAMDYWGQGTLVTVSS

SEQ ID NO: 24 - protein, 121 aa, synthetic construct
QVQLVESGGGVVQPGRSLRLSCAASGFSLTSYGVTWVRQSPGKGLEWVAVIWGDGSTNYHSGLRSRLTISRDNSKNTLYLEMNSLRTEDTATYYCAKPIYYDFDDDAMDYWGQGTKVTVSS

SEQ ID NO: 25 - protein, 121 aa, synthetic construct
QVQLQESGPGLVKPSETLSLTCTVSGFSLTSYGVTWIRQPPGKGLEWIGVIWGDGSTNYHSGLRSRVTISVDTSKNQFSLKLSSVTAADTAVYYCAKPIYYDFDDDAMDYWGQGTSVTVSS

SEQ ID NO: 26 - protein, 107 aa, synthetic construct
  VARIANT 55: note = X is A, R, N, D, Q, E, G, H, I, L, K, M, F, S, T, W, Y, or V
EIVMTQSPSSLSASVGDRVTITCKASQNVGTYVAWFQQKPGKAPKSLIYSASYRXSGVPSKFSGSGSGTDFTLTISSLQPEDFATYYCHQYNNYPLTFGQGTKLEIK

SEQ ID NO: 27 - protein, 107 aa, synthetic construct
  VARIANT 55: note = X is A, R, N, D, Q, E, G, H, I, L, K, M, F, S, T, W, Y, or V
DIQMTQSPSSLSASVGDRVTITCKASQNVGTYVAWYQQKPGKAPKLLIYSASYRXSGVPSRFSGSGSGTEFTLTISSLQPDDFTTYYCHQYNNYPLTFGQGTKVEIK

SEQ ID NO: 28 - protein, 107 aa, synthetic construct
  VARIANT 55: note = X is A, R, N, D, Q, E, G, H, I, L, K, M, F, S, T, W, Y, or V
DIVMTQSPSSLSLSPGDRATLSCKASQNVGTYVAWYQQKPGQAPRLLIYSASYRXSGIPARFSGSGSGTDFTLTISSLQSEDFAVYYCHQYNNYPLTFGGGTKVEIK

SEQ ID NO: 29 - protein, 107 aa, synthetic construct
EIVMTQSPSSLSASVGDRVTITCKASQNVGTYVAWFQQKPGKAPKSLIYSASYRCSGVPSKFSGSGSGTDFTLTISSLQPEDFATYYCHQYNNYPLTFGQGTKLEIK

SEQ ID NO: 30 - protein, 107 aa, synthetic construct
DIQMTQSPSSLSASVGDRVTITCKASQNVGTYVAWYQQKPGKAPKLLIYSASYRCSGVPSRFSGSGSGTEFTLTISSLQPDDFTTYYCHQYNNYPLTFGQGTKVEIK

SEQ ID NO: 31 - protein, 107 aa, synthetic construct
DIVMTQSPSSLSLSPGDRATLSCKASQNVGTYVAWYQQKPGQAPRLLIYSASYRCSGIPARFSGSGSGTDFTLTISSLQSEDFAVYYCHQYNNYPLTFGGGTKVEIK

SEQ ID NO: 32 - protein, 107 aa, synthetic construct
  VARIANT 55: note = X is A, R, N, D, Q, E, G, H, I, L, K, M, F, S, T, W, Y, or V
EIVLTQSPSSLSASVGDRVTITCKASQNVGTYVAWFQQKPGKAPKSLIYSASYRXSGVPSKFSGSGSGTDFTLTISSLQPEDFATYYCHQYNNYPLTFGQGTKLEIK

SEQ ID NO: 33 - protein, 107 aa, synthetic construct
  VARIANT 55: note = X is A, R, N, D, Q, E, G, H, I, L, K, M, F, S, T, W, Y, or V
DIQMTQSPSSLSASVGDRVTITCKASQNVGTYVAWFQQRPGKAPKSLIYSASYRXSGVPSKFSGSGSGTDFTLTINSLQPEDFATYYCHQYNNYPLTFGQGTKVEIK

SEQ ID NO: 34 - protein, 107 aa, synthetic construct
  VARIANT 55: note = X is A, R, N, D, Q, E, G, H, I, L, K, M, F, S, T, W, Y, or V
DIQLTQSPSTLSASVGDRVTITCKASQNVGTYVAWYQQKPGKAPKLLIYSASYRXSGVPSRFSGSGSGTEFTLTISSLQPDDFTTYYCHQYNNYPLTFGQGTKVEIK

SEQ ID NO: 35 - protein, 107 aa, synthetic construct
  VARIANT 55: note = X is A, R, N, D, Q, E, G, H, I, L, K, M, F, S, T, W, Y, or V
DIVMTQSPATLSLSPGDRATLSCKASQNVGTYVAWYQQKPGQAPRLLIYSASYRXSGIPARFSGSGSGTDFTLTISSLQSEDFAVYYCHQYNNYPLTFGGGTKVEIK

SEQ ID NO: 36 - protein, 244 aa, synthetic construct
PLPKPSLQALPSSLVPLEKPVTLRCQGPPGVDLYRLEKLSSSRYQDQAVLFIPAMKRSLAGRYRCSYQNGSLWSLPSDQLELVATGVFAKPSLSAQPGPAVSSGGDVTLQCQTRYGFDQFALYKEGDPAPYKNPERWYRASFPIITVTAAHSGTYRCYSFSSRDPYLWSAPSDPLELVVTGTSVTPSRLPTEPPSPVAEFSEATAELTVSFTNEVFTTETSRSITASPKESDSPAGPARQYYTK

SEQ ID NO: 37 - protein, 234 aa, synthetic construct
MVSSAQFLGLLLLCFQGTRCDIVMTQSQKFMSTSVGDRVSVTCKASQNVGTYVAWFQQKPGQSPKTLIYSASYRCSGVPDRFTGSGSGTDFTLTISNVQSDDLAEYFCHQYNNYPLTFGAGTKLELRRTVAAPSVFIFPPSDEQLKSGTASVVCLLNNFYPREAKVQWKVDNALQSGNSQESVTEQDSKDSTYSLSSTLTLSKADYEKHKVYACEVTHQGLSSPVTKSFNRGEC

SEQ ID NO: 38 - protein, 234 aa, synthetic construct
MVSSAQFLGLLLLCFQGTRCEIVLTQSPSSLSASVGDRVTITCKASQNVGTYVAWFQQKPGKAPKSLIYSASYRCSGVPSKFSGSGSGTDFTLTISSLQPEDFATYYCHQYNNYPLTFGQGTKLEIKRTVAAPSVFIFPPSDEQLKSGTASVVCLLNNFYPREAKVQWKVDNALQSGNSQESVTEQDSKDSTYSLSSTLTLSKADYEKHKVYACEVTHQGLSSPVTKSFNRGEC

SEQ ID NO: 39 - protein, 234 aa, synthetic construct
MVSSAQFLGLLLLCFQGTRCDIQMTQSPSSLSASVGDRVTITCKASQNVGTYVAWFQQRPGKAPKSLIYSASYRCSGVPSKFSGSGSGTDFTLTINSLQPEDFATYYCHQYNNYPLTFGQGTKVEIKRTVAAPSVFIFPPSDEQLKSGTASVVCLLNNFYPREAKVQWKVDNALQSGNSQESVTEQDSKDSTYSLSSTLTLSKADYEKHKVYACEVTHQGLSSPVTKSFNRGEC

SEQ ID NO: 40 - protein, 234 aa, synthetic construct
MVSSAQFLGLLLLCFQGTRCDIQLTQSPSTLSASVGDRVTITCKASQNVGTYVAWYQQKPGKAPKLLIYSASYRCSGVPSRFSGSGSGTEFTLTISSLQPDDFTTYYCHQYNNYPLTFGQGTKVEIKRTVAAPSVFIFPPSDEQLKSGTASVVCLLNNFYPREAKVQWKVDNALQSGNSQESVTEQDSKDSTYSLSSTLTLSKADYEKHKVYACEVTHQGLSSPVTKSFNRGEC

SEQ ID NO: 41 - protein, 234 aa, synthetic construct
MVSSAQFLGLLLLCFQGTRCDIVMTQSPATLSLSPGDRATLSCKASQNVGTYVAWYQQKPGQAPRLLIYSASYRCSGIPARFSGSGSGTDFTLTISSLQSEDFAVYYCHQYNNYPLTFGGGTKVEIKRTVAAPSVFIFPPSDEQLKSGTASVVCLLNNFYPREAKVQWKVDNALQSGNSQESVTEQDSKDSTYSLSSTLTLSKADYEKHKVYACEVTHQGLSSPVTKSFNRGEC

SEQ ID NO: 42 - protein, 214 aa, synthetic construct
DIQMTQSPSSLSASVGDRVTITCKASQNVGTYVAWFQQRPGKAPKSLIYSASYRCSGVPSKFSGSGSGTDFTLTINSLQPEDFATYYCHQYNNYPLTFGQGTKVEIKRTVAAPSVFIFPPSDEQLKSGTASVVCLLNNFYPREAKVQWKVDNALQSGNSQESVTEQDSKDSTYSLSSTLTLSKADYEKHKVYACEVTHQGLSSPVTKSFNRGEC

SEQ ID NO: 43 - protein, 247 aa, synthetic construct
MGWTLVFLFLLSVTAGVHSQVQLKESGPGLVQPSQSLSITCTVSGFSLTSYGVTWVRQPPGKGLEWLGVIWGDGSTNYHSGLRSRLSISRDDSKSQVFLKLNSLQTDDTATYYCAKPIYYDFDDDAMDYWGQGTSVTVSSASTKGPSVFPLAPSSKSTSGGTAALGCLVKDYFPEPVTVSWNSGALTSGVHTFPAVLQSSGLYSLSSVVTVPSSSLGTQTYICNVNHKPSNTKVDKKVEPKSCDKTH

SEQ ID NO: 44 - protein, 247 aa, synthetic construct
MGWTLVFLFLLSVTAGVHSQVQLQESGPGLVKPSETLSLTCTASGFSLTSYGVTWIRQPPGKGLEWIGVIWGDGSTNYHSGLRSRVTISVDTSKSQFSLKLSSVTAADTAVYYCAKPIYYDFDDDAMDYWGQGTLVTVSSASTKGPSVFPLAPSSKSTSGGTAALGCLVKDYFPEPVTVSWNSGALTSGVHTFPAVLQSSGLYSLSSVVTVPSSSLGTQTYICNVNHKPSNTKVDKKVEPKSCDKTH

SEQ ID NO: 45 - protein, 247 aa, synthetic construct
MGWTLVFLFLLSVTAGVHSEVQLVESGPGLVKPSETLSLTCTVSGFSLTSYGVTWIRQPPGKGLEWIGVIWGDGSTNYHSGLRSRVTISVDTSKNQFSLKLSSVTAADTAVYYCAKPIYYDFDDDAMDYWGQGTLVTVSSASTKGPSVFPLAPSSKSTSGGTAALGCLVKDYFPEPVTVSWNSGALTSGVHTFPAVLQSSGLYSLSSVVTVPSSSLGTQTYICNVNHKPSNTKVDKKVEPKSCDKTH

SEQ ID NO: 46 - protein, 247 aa, synthetic construct
MGWTLVFLFLLSVTAGVHSQVQLVESGGGVVQPGRSLRLSCVASGFSLTSYGVTWVRQAPGKGLEWVAVIWGDGSTNYHSGLRSRFTISRDNSKNTMFLQMNSLRADDTAVYYCAKPIYYDFDDDAMDYWGQGTLVTVSSASTKGPSVFPLAPSSKSTSGGTAALGCLVKDYFPEPVTVSWNSGALTSGVHTFPAVLQSSGLYSLSSVVTVPSSSLGTQTYICNVNHKPSNTKVDKKVEPKSCDKTH

SEQ ID NO: 47 - protein, 247 aa, synthetic construct
MGWTLVFLFLLSVTAGVHSQVQLVESGGGVVQPGRSLRLSCAASGFSLTSYGVTWVRQSPGKGLEWVAVIWGDGSTNYHSGLRSRLTISRDNSKNTLYLEMNSLRTEDTATYYCAKPIYYDFDDDAMDYWGQGTKVTVSSASTKGPSVFPLAPSSKSTSGGTAALGCLVKDYFPEPVTVSWNSGALTSGVHTFPAVLQSSGLYSLSSVVTVPSSSLGTQTYICNVNHKPSNTKVDKKVEPKSCDKTH

SEQ ID NO: 48 - protein, 247 aa, synthetic construct
MGWTLVFLFLLSVTAGVHSQVQLQESGPGLVKPSETLSLTCTVSGFSLTSYGVTWIRQPPGKGLEWIGVIWGDGSTNYHSGLRSRVTISVDTSKNQFSLKLSSVTAADTAVYYCAKPIYYDFDDDAMDYWGQGTSVTVSSASTKGPSVFPLAPSSKSTSGGTAALGCLVKDYFPEPVTVSWNSGALTSGVHTFPAVLQSSGLYSLSSVVTVPSSSLGTQTYICNVNHKPSNTKVDKKVEPKSCDKTH

SEQ ID NO: 49 - protein, 234 aa, synthetic construct
MVSSAQFLGLLLLCFQGTRCEIVMTQSPSSLSASVGDRVTITCKASQNVGTYVAWFQQKPGKAPKSLIYSASYRCSGVPSKFSGSGSGTDFTLTISSLQPEDFATYYCHQYNNYPLTFGQGTKLEIKRTVAAPSVFIFPPSDEQLKSGTASVVCLLNNFYPREAKVQWKVDNALQSGNSQESVTEQDSKDSTYSLSSTLTLSKADYEKHKVYACEVTHQGLSSPVTKSFNRGEC

SEQ ID NO: 50 - protein, 234 aa, synthetic construct
MVSSAQFLGLLLLCFQGTRCDIQMTQSPSSLSASVGDRVTITCKASQNVGTYVAWYQQKPGKAPKLLIYSASYRCSGVPSRFSGSGSGTEFTLTISSLQPDDFTTYYCHQYNNYPLTFGQGTKVEIKRTVAAPSVFIFPPSDEQLKSGTASVVCLLNNFYPREAKVQWKVDNALQSGNSQESVTEQDSKDSTYSLSSTLTLSKADYEKHKVYACEVTHQGLSSPVTKSFNRGEC

SEQ ID NO: 51 - protein, 234 aa, synthetic construct
MVSSAQFLGLLLLCFQGTRCDIVMTQSPSSLSLSPGDRATLSCKASQNVGTYVAWYQQKPGQAPRLLIYSASYRCSGIPARFSGSGSGTDFTLTISSLQSEDFAVYYCHQYNNYPLTFGGGTKVEIKRTVAAPSVFIFPPSDEQLKSGTASVVCLLNNFYPREAKVQWKVDNALQSGNSQESVTEQDSKDSTYSLSSTLTLSKADYEKHKVYACEVTHQGLSSPVTKSFNRGEC

SEQ ID NO: 52 - protein, 234 aa, synthetic construct
  VARIANT 75: note = X is A, R, N, D, Q, E, G, H, I, L, K, M, F, S, T, W, Y, or V
MVSSAQFLGLLLLCFQGTRCEIVMTQSPSSLSASVGDRVTITCKASQNVGTYVAWFQQKPGKAPKSLIYSASYRXSGVPSKFSGSGSGTDFTLTISSLQPEDFATYYCHQYNNYPLTFGQGTKLEIKRTVAAPSVFIFPPSDEQLKSGTASVVCLLNNFYPREAKVQWKVDNALQSGNSQESVTEQDSKDSTYSLSSTLTLSKADYEKHKVYACEVTHQGLSSPVTKSFNRGEC

SEQ ID NO: 53 - protein, 234 aa, synthetic construct
  VARIANT 75: note = X is A, R, N, D, Q, E, G, H, I, L, K, M, F, S, T, W, Y, or V
MVSSAQFLGLLLLCFQGTRCDIQMTQSPSSLSASVGDRVTITCKASQNVGTYVAWYQQKPGKAPKLLIYSASYRXSGVPSRFSGSGSGTEFTLTISSLQPDDFTTYYCHQYNNYPLTFGQGTKVEIKRTVAAPSVFIFPPSDEQLKSGTASVVCLLNNFYPREAKVQWKVDNALQSGNSQESVTEQDSKDSTYSLSSTLTLSKADYEKHKVYACEVTHQGLSSPVTKSFNRGEC

SEQ ID NO: 54 - protein, 234 aa, synthetic construct
  VARIANT 75: note = X is A, R, N, D, Q, E, G, H, I, L, K, M, F, S, T, W, Y, or V
MVSSAQFLGLLLLCFQGTRCDIVMTQSPSSLSLSPGDRATLSCKASQNVGTYVAWYQQKPGQAPRLLIYSASYRXSGIPARFSGSGSGTDFTLTISSLQSEDFAVYYCHQYNNYPLTFGGGTKVEIKRTVAAPSVFIFPPSDEQLKSGTASVVCLLNNFYPREAKVQWKVDNALQSGNSQESVTEQDSKDSTYSLSSTLTLSKADYEKHKVYACEVTHQGLSSPVTKSFNRGEC

SEQ ID NO: 55 - protein, 234 aa, synthetic construct
  VARIANT 75: note = X is A, R, N, D, Q, E, G, H, I, L, K, M, F, S, T, W, Y, or V
MVSSAQFLGLLLLCFQGTRCEIVLTQSPSSLSASVGDRVTITCKASQNVGTYVAWFQQKPGKAPKSLIYSASYRXSGVPSKFSGSGSGTDFTLTISSLQPEDFATYYCHQYNNYPLTFGQGTKLEIKRTVAAPSVFIFPPSDEQLKSGTASVVCLLNNFYPREAKVQWKVDNALQSGNSQESVTEQDSKDSTYSLSSTLTLSKADYEKHKVYACEVTHQGLSSPVTKSFNRGEC

SEQ ID NO: 56 - protein, 234 aa, synthetic construct
  VARIANT 75: note = X is A, R, N, D, Q, E, G, H, I, L, K, M, F, S, T, W, Y, or V
MVSSAQFLGLLLLCFQGTRCDIQMTQSPSSLSASVGDRVTITCKASQNVGTYVAWFQQRPGKAPKSLIYSASYRXSGVPSKFSGSGSGTDFTLTINSLQPEDFATYYCHQYNNYPLTFGQGTKVEIKRTVAAPSVFIFPPSDEQLKSGTASVVCLLNNFYPREAKVQWKVDNALQSGNSQESVTEQDSKDSTYSLSSTLTLSKADYEKHKVYACEVTHQGLSSPVTKSFNRGEC

SEQ ID NO: 57 - protein, 234 aa, synthetic construct
  VARIANT 75: note = X is A, R, N, D, Q, E, G, H, I, L, K, M, F, S, T, W, Y, or V
MVSSAQFLGLLLLCFQGTRCDIQLTQSPSTLSASVGDRVTITCKASQNVGTYVAWYQQKPGKAPKLLIYSASYRXSGVPSRFSGSGSGTEFTLTISSLQPDDFTTYYCHQYNNYPLTFGQGTKVEIKRTVAAPSVFIFPPSDEQLKSGTASVVCLLNNFYPREAKVQWKVDNALQSGNSQESVTEQDSKDSTYSLSSTLTLSKADYEKHKVYACEVTHQGLSSPVTKSFNRGEC

SEQ ID NO: 58 - protein, 234 aa, synthetic construct
  VARIANT 75: note = X is A, R, N, D, Q, E, G, H, I, L, K, M, F, S, T, W, Y, or V
MVSSAQFLGLLLLCFQGTRCDIVMTQSPATLSLSPGDRATLSCKASQNVGTYVAWYQQKPGQAPRLLIYSASYRXSGIPARFSGSGSGTDFTLTISSLQSEDFAVYYCHQYNNYPLTFGGGTKVEIKRTVAAPSVFIFPPSDEQLKSGTASVVCLLNNFYPREAKVQWKVDNALQSGNSQESVTEQDSKDSTYSLSSTLTLSKADYEKHKVYACEVTHQGLSSPVTKSFNRGEC

SEQ ID NO: 59 - protein, 228 aa, synthetic construct
QVQLQESGPGLVKPSETLSLTCTASGFSLTSYGVTWIRQPPGKGLEWIGVIWGDGSTNYHSGLRSRVTISVDTSKSQFSLKLSSVTAADTAVYYCAKPIYYDFDDDAMDYWGQGTLVTVSSASTKGPSVFPLAPSSKSTSGGTAALGCLVKDYFPEPVTVSWNSGALTSGVHTFPAVLQSSGLYSLSSVVTVPSSSLGTQTYICNVNHKPSNTKVDKKVEPKSCDKTH

SEQ ID NO: 60 - protein, 107 aa, synthetic construct [sequence omitted]

SEQ ID NO: 61 - protein, 107 aa, synthetic construct
ASTKGPSVFPLAPSSKSTSGGTAALGCLVKDYFPEPVTVSWNSGALTSGVHTFPAVLQSSGLYSLSSVVTVPSSSLGTQTYICNVNHKPSNTKVDKKVEPKSCDKTH

SEQ ID NO: 62 - protein, 20 aa, synthetic construct
MVSSAQFLGLLLLCFQGTRC

SEQ ID NO: 63 - protein, 19 aa, synthetic construct
MGWTLVFLFLLSVTAGVHS